European Patent Specification EP 3 411 406 B1, published April 9, 2025. Title: MULTISPECIFIC ANTIGEN-BINDING MOLECULE WITH IMPROVED INTERNALIZATION CHARACTERISTICS. Applicant: Genmab A/S. The sequence listing filed with the application follows.

SEQUENCE LISTING (12 sequences)

SEQ ID NO: 1 - protein, 120 aa, Homo Sapiens
EVQLQQSGPELVKPGASVKMSCKASGYTFTSYVMHWVRQTPGQGLEWIGYITPYNDGTKYNEKFKGKATLTSDKSSSTAYMELSSLTSEDSAVYYCVGGDNYYYAMDYWGQGTSVTVSAA

SEQ ID NO: 2 - protein, 8 aa, Homo Sapiens
GYTFTSYV

SEQ ID NO: 3 - protein, 8 aa, Homo Sapiens
ITPYNDGT

SEQ ID NO: 4 - protein, 12 aa, Homo Sapiens
VGGDNYYYAMDY

SEQ ID NO: 5 - protein, 114 aa, Homo Sapiens
NIMVTQSPSSLAVSAGEKVTMSCKSSQSVLYSSNQKNYLAWYQQKPGQSPKLLIYWASTRVSGVPDRFTGSGSGTDFTLTISRVQAEDLAVYYCHQYFSSFTFGSGTKLEIKRT

SEQ ID NO: 6 - protein, 12 aa, Homo Sapiens
QSVLYSSNQKNY

SEQ ID NO: 7 - protein, 3 aa, Homo Sapiens
WAS

SEQ ID NO: 8 - protein, 8 aa, Homo Sapiens
HQYFSSFT

SEQ ID NO: 9 - protein, 12 aa, Homo Sapiens
QSVLYSSHQKNY

SEQ ID NO: 10 - protein, 8 aa, Homo Sapiens
IHPYNDGT

SEQ ID NO: 11 - protein, 8 aa, Homo Sapiens
ITHYNDGT

SEQ ID NO: 12 - protein, 8 aa, Homo Sapiens
ITPYHDGT